European Patent Application EP 4 306 638 A1, published January 17, 2024. Title: 7-Keto-LCA에서 우르소데옥시콜산으로의 전환율을 증진시키는 루미노코쿠스 나버스 균주 유래 7-beta-HSDH의 변이체 및 이를 이용한 우르소데옥시콜산 생산방법. Applicant: 에이스바이오팜 주식회사. Application KR. The sequence listing filed with the application follows.

SEQUENCE LISTING (14 sequences)

SEQ ID NO: 1 - protein, 789 aa, Artificial Sequence
METTHRLEUARGGLULYSTYRGLYGLUTRPGLYILEILELEUGLYALATHRGLUGLYVALGLYLYSALAPHECYSGLUARGLEUALALYSGLUGLYMETASNVALVALMETVALGLYARGARGGLUGLULYSLEULYSGLULEUGLYGLUGLULEULYSASNTHRTYRGLUILEASPTYRLYSVALVALLYSALAASPPHESERLEUPROASPALATHRASPLYSILEPHEALAALATHRGLUASNLEUASPMETGLYPHEMETALATYRVALALACYSLEUHISSERPHEGLYLYSILEGLNASPTHRPROTRPGLULYSHISGLUALAMETILEASNVALASNVALVALTHRPHEMETLYSCYSPHETYRHISTYRMETLYSILEPHEALAALAGLNASPARGGLYALAVALILEASNVALSERSERMETTHRGLYILESERSERSERPROTRPASNGLYGLNTYRGLYALAGLYLYSALAPHEILELEULYSMETTHRGLUALAVALALACYSGLUTHRGLULYSTHRASNVALASPVALGLUVALILETHRLEUGLYTHRVALLEUTHRPROSERLEULEUSERASNLEUPROGLYGLYPROGLNGLYGLUALAVALMETLYSILEALALEUTHRPROGLUGLUVALVALASPGLUALAPHEGLULYSLEUGLYLYSGLULEUSERVALILESERGLYGLUARGASNLYSALASERVALHISASPTRPLYSALAASNHISTHRGLUASPGLUTYRILEARGTYRMETGLYSERPHETYRGLNGLU

SEQ ID NO: 2 - DNA, 792 bp, Artificial Sequence
  source 1..792: mol_type = genomic DNA
atgactttacgcgagaaatacggtgagtggggaattattcttggtgctacagagggcgtaggcaaggccttctgcgagcgtttagcgaaggaggggatgaatgttgtcatggtaggacgccgcgaggaaaaattgaaggaattaggagaagagcttaagaacacctatgaaatcgactataaagttgttaaggccgacttttctttgcccgacgcgaccgataaaattttcgcggcgactgaaaatttggacatgggatttatggcctatgttgcatgcttgcactcgtttggtaagattcaagacactccctgggagaagcacgaagcaatgattaacgtgaatgtcgtcacgttcttgaaatgctttcaccactatatgcgtatttttgcggcgcaggatcgtggagcggtaattaacgtgtcttccatgacggggattagctctagcccatggaatggccaatacggcgctggtaaagcatttattcttaagatgaccgaagccgtggcatgtgaatgcgagggaaccggagtggacgtggaggtaattacgctgggaaccacccttacgccgtcacttttgtccaacctgccgggcgggccacaaggagaagctgtaatgaaaattgcattgactcccgaagagtgcgtagatgaggcttttgaaaagttgggaaaagaattgtctgtgattgcaggccaacgcaacaaagactcagttcatgactggaaagctaaccacactgaggacgaatacatccgctacatgggctccttctaccgtgattaa

SEQ ID NO: 3 - protein, 789 aa, Ruminococcus gnavus
METTHRLEUARGGLULYSTYRGLYGLUTRPGLYILEILELEUGLYALATHRGLUGLYVALGLYLYSALAPHECYSGLUARGLEUALALYSGLUGLYMETASNVALVALMETVALGLYARGARGGLUGLULYSLEULYSGLULEUGLYGLUGLULEULYSASNTHRTYRGLUILEASPTYRLYSVALVALLYSALAASPPHESERLEUPROASPALATHRASPLYSILEPHEALAALATHRGLUASNLEUASPMETGLYPHEMETALATYRVALALACYSLEUHISSERPHEGLYLYSILEGLNASPTHRPROTRPGLULYSHISGLUALAMETILEASNVALASNVALVALTHRPHEMETLYSCYSPHETYRHISTYRMETLYSILEPHEALAALAGLNASPARGGLYALAVALILEASNVALSERSERMETTHRGLYILESERSERSERPROTRPASNGLYGLNTYRGLYALAGLYLYSALAPHEILELEULYSMETTHRGLUALAVALALACYSGLUTHRGLULYSTHRASNVALASPVALGLUVALILETHRLEUGLYTHRVALLEUTHRPROSERLEULEUSERASNLEUPROGLYGLYPROGLNGLYGLUALAMETMETLYSTHRALAGLNTHRPROGLUGLUVALVALASPGLUALAPHEGLULYSLEUGLYLYSGLULEUSERVALILESERGLYGLUARGASNLYSALASERVALHISASPTRPLYSALAASNHISTHRGLUASPASPTYRILEARGTYRMETGLYSERPHETYRGLNGLU

SEQ ID NO: 4 - DNA, 792 bp, Ruminococcus gnavus
  source 1..792: mol_type = genomic DNA
atgacattgagagaaaaatatggagaatggggaattattttaggcgctactgaaggtgtcggaaaagcattttgtgaaaggcttgccaaagaaggtatgaatgtcgtaatggtcggacgccgtgaagaaaaattaaaagagctcggtgaggaactaaaaaacacttatgagattgattataaagtcgtaaaagcagacttttcgctgccagatgctactgacaaaatttttgctgcaacagaaaatctggatatgggatttatggcctatgtagcctgcttacactcttttggcaaaatccaggatacaccttgggaaaagcatgaggcaatgatcaacgtaaacgttgttacatttatgaaatgcttctatcactatatgaaaatctttgctgcacaggatcgcggtgctgtcatcaacgtatcttctatgactggaatttccagttcaccatggaatggccaatatggtgcaggaaaggcattcattttaaaaatgacagaggctgttgcctgtgaaacggaaaagaccaatgttgatgtggaagtcatcactttgggaactgtgctgacaccaagtcttttaagcaacctgcctggcggaccacagggggaagctatgatgaagactgctcaaacaccggaagaagttgtggacgaagcttttgaaaaattaggaaaagaactgtctgtcatttccggagagcgtaataaagccagcgtccatgactggaaagcgaatcatacagaagatgactatatccgctatatgggatctttctatcaagaataa

SEQ ID NO: 5 - DNA, 38 bp, Artificial Sequence
  source 1..38: mol_type = other DNA
ataaggagatataccatgaatttgcgtgagaaatacgg

SEQ ID NO: 6 - DNA, 41 bp, Artificial Sequence
  source 1..41: mol_type = other DNA
ctcgaattcggatccttaatctctgtaaaagctacccatgt

SEQ ID NO: 7 - DNA, 30 bp, Artificial Sequence
  source 1..30: mol_type = other DNA
ataaggagatataccatgacattgagagaa

SEQ ID NO: 8 - DNA, 30 bp, Artificial Sequence
  source 1..30: mol_type = other DNA
gaattcggatccttattattcttgatagaa

SEQ ID NO: 9 - DNA, 49 bp, Artificial Sequence
  source 1..49: mol_type = other DNA
cattatacgagccgatgattaattgtcaaatttcgcgggatcgagatcg

SEQ ID NO: 10 - DNA, 53 bp, Artificial Sequence
  source 1..53: mol_type = other DNA
ttgacaattaatcatcggctcgtataatgggaattgtgagcggataacaattc

SEQ ID NO: 11 - DNA, 30 bp, Artificial Sequence
  source 1..30: mol_type = other DNA
acgaattgttagacattagaaaaactcatc

SEQ ID NO: 12 - DNA, 30 bp, Artificial Sequence
  source 1..30: mol_type = other DNA
ttgaaaaaggaagagatgagccatattcaa

SEQ ID NO: 13 - DNA, 27 bp, Artificial Sequence
  source 1..27: mol_type = other DNA
actcttcctttttcaatattattgaag

SEQ ID NO: 14 - DNA, 27 bp, Artificial Sequence
  source 1..27: mol_type = other DNA
tgtctaacaattcgttcaagccgaggg